European Patent Application EP 4 538 362 A1, published April 16, 2025. Title: Microorganisms with improved productivity of 3'-sialyllactose and method of producing 3'-sialyllactose. Applicant: 協和発酵バイオ株式会社. The sequence listing filed with the application follows.

SEQUENCE LISTING (56 sequences)

SEQ ID NO: 1 - DNA, 1137 bp, Neisseria lactamica
  source 1..1137: mol_type = genomic DNA; strain = ATCC23970
atgggcctgaagaaagcgtgcctgaccgttctgtgtctgatcgtcttttgcttcggcatcttttatacgttcgatcgtgtgaaccagggtgaacgcaatgctgttagcctgctgaaagacaaactgtttaacgaagaaggcgaaccggtgaatctgatcttctgttataccattctgcagatgaaagttgcagaacgtattatggctcaacatccgggtgaacgcttttacgtggttctgatgtctgaaaaccgtaacgaaaaatacgattactacttcaaccaaatcaaagacaaagcagaacgcgcttatttcttttatctgccgtacggtctgaacaaaagcttcaacttcatcccgaccatggcagaactgaaagtcaaatctatgctgctgccgaaagtgaaacgtatctacctggcgtcactggaaaaagtgtcgattgcggcctttctgtcaacctatccggatgccgaaatcaaaaccttcgatgacggcacgaacaatctgattcaggaaagctcttatctgggcgatgaattttcggttaacggtacgatcaaacgtaatttcgcccgcatgatgatcggtgattggagtattgcgaaaacccgcaacgcctccgacgaacattacacgatcttcaaaggcctgaaaaacatcatggatgacggtcgtcgcaaaatgacctatctgccgctgttcgatgcaagcgaactgaaagctggcgacgaaaccggcggtacggtccgtattctgctgggttcaccggataaagaaatgaaagaaatctcggaaaaagcagctaaaaacttcaaaatccagtacgttgcgccgcacccgcgccaaacctatggtctgagcggtgttaccacgctgaactctccgtacgtcattgaagattacatcctgcgtgaaattaagaaaaacccgcatacccgctacgaaatctatacgtttttcagcggcgcggccctgacgatgaaagattttccgaacgtccacgtgtatgcgctgaaaccggccagtctgccggaagactactggctgaaaccggtgtatgccctgtttacccagtccggcattccgatcctgacgttcgatgacaaaaaccaaagttacggtaaatccaaataa

SEQ ID NO: 2 - protein, 378 aa, Neisseria lactamica
  source 1..378: note = strain, ATCC23970
MGLKKACLTVLCLIVFCFGIFYTFDRVNQGERNAVSLLKDKLFNEEGEPVNLIFCYTILQMKVAERIMAQHPGERFYVVLMSENRNEKYDYYFNQIKDKAERAYFFYLPYGLNKSFNFIPTMAELKVKSMLLPKVKRIYLASLEKVSIAAFLSTYPDAEIKTFDDGTNNLIQESSYLGDEFSVNGTIKRNFARMMIGDWSIAKTRNASDEHYTIFKGLKNIMDDGRRKMTYLPLFDASELKAGDETGGTVRILLGSPDKEMKEISEKAAKNFKIQYVAPHPRQTYGLSGVTTLNSPYVIEDYILREIKKNPHTRYEIYTFFSGAALTMKDFPNVHVYALKPASLPEDYWLKPVYALFTQSGIPILTFDDKNQSYGKSK

SEQ ID NO: 3 - DNA, 1080 bp, synthetic construct
  misc_feature 1..1080: note = Base sequence of tNlsiaT delta N20AA
  source 1..1080: mol_type = other DNA
atgttttatacgttcgatcgtgtgaaccagggtgaacgcaatgctgttagcctgctgaaagacaaactgtttaacgaagaaggcgaaccggtgaatctgatcttctgttataccattctgcagatgaaagttgcagaacgtattatggctcaacatccgggtgaacgcttttacgtggttctgatgtctgaaaaccgtaacgaaaaatacgattactacttcaaccaaatcaaagacaaagcagaacgcgcttatttcttttatctgccgtacggtctgaacaaaagcttcaacttcatcccgaccatggcagaactgaaagtcaaatctatgctgctgccgaaagtgaaacgtatctacctggcgtcactggaaaaagtgtcgattgcggcctttctgtcaacctatccggatgccgaaatcaaaaccttcgatgacggcacgaacaatctgattcaggaaagctcttatctgggcgatgaattttcggttaacggtacgatcaaacgtaatttcgcccgcatgatgatcggtgattggagtattgcgaaaacccgcaacgcctccgacgaacattacacgatcttcaaaggcctgaaaaacatcatggatgacggtcgtcgcaaaatgacctatctgccgctgttcgatgcaagcgaactgaaagctggcgacgaaaccggcggtacggtccgtattctgctgggttcaccggataaagaaatgaaagaaatctcggaaaaagcagctaaaaacttcaaaatccagtacgttgcgccgcacccgcgccaaacctatggtctgagcggtgttaccacgctgaactctccgtacgtcattgaagattacatcctgcgtgaaattaagaaaaacccgcatacccgctacgaaatctatacgtttttcagcggcgcggccctgacgatgaaagattttccgaacgtccacgtgtatgcgctgaaaccggccagtctgccggaagactactggctgaaaccggtgtatgccctgtttacccagtccggcattccgatcctgacgttcgatgacaaaaaccaaagttacggtaaatccaaataa

SEQ ID NO: 4 - protein, 359 aa, synthetic construct
  REGION 1..359: note = Amino acid sequence of tNlsiaT delta N20AA
MFYTFDRVNQGERNAVSLLKDKLFNEEGEPVNLIFCYTILQMKVAERIMAQHPGERFYVVLMSENRNEKYDYYFNQIKDKAERAYFFYLPYGLNKSFNFIPTMAELKVKSMLLPKVKRIYLASLEKVSIAAFLSTYPDAEIKTFDDGTNNLIQESSYLGDEFSVNGTIKRNFARMMIGDWSIAKTRNASDEHYTIFKGLKNIMDDGRRKMTYLPLFDASELKAGDETGGTVRILLGSPDKEMKEISEKAAKNFKIQYVAPHPRQTYGLSGVTTLNSPYVIEDYILREIKKNPHTRYEIYTFFSGAALTMKDFPNVHVYALKPASLPEDYWLKPVYALFTQSGIPILTFDDKNQSYGKSK

SEQ ID NO: 5 - DNA, 1071 bp, synthetic construct
  misc_feature 1..1071: note = Base sequence of tNlsiaT delta N23AA
  source 1..1071: mol_type = other DNA
atgttcgatcgtgtgaaccagggtgaacgcaatgctgttagcctgctgaaagacaaactgtttaacgaagaaggcgaaccggtgaatctgatcttctgttataccattctgcagatgaaagttgcagaacgtattatggctcaacatccgggtgaacgcttttacgtggttctgatgtctgaaaaccgtaacgaaaaatacgattactacttcaaccaaatcaaagacaaagcagaacgcgcttatttcttttatctgccgtacggtctgaacaaaagcttcaacttcatcccgaccatggcagaactgaaagtcaaatctatgctgctgccgaaagtgaaacgtatctacctggcgtcactggaaaaagtgtcgattgcggcctttctgtcaacctatccggatgccgaaatcaaaaccttcgatgacggcacgaacaatctgattcaggaaagctcttatctgggcgatgaattttcggttaacggtacgatcaaacgtaatttcgcccgcatgatgatcggtgattggagtattgcgaaaacccgcaacgcctccgacgaacattacacgatcttcaaaggcctgaaaaacatcatggatgacggtcgtcgcaaaatgacctatctgccgctgttcgatgcaagcgaactgaaagctggcgacgaaaccggcggtacggtccgtattctgctgggttcaccggataaagaaatgaaagaaatctcggaaaaagcagctaaaaacttcaaaatccagtacgttgcgccgcacccgcgccaaacctatggtctgagcggtgttaccacgctgaactctccgtacgtcattgaagattacatcctgcgtgaaattaagaaaaacccgcatacccgctacgaaatctatacgtttttcagcggcgcggccctgacgatgaaagattttccgaacgtccacgtgtatgcgctgaaaccggccagtctgccggaagactactggctgaaaccggtgtatgccctgtttacccagtccggcattccgatcctgacgttcgatgacaaaaaccaaagttacggtaaatccaaataa

SEQ ID NO: 6 - protein, 356 aa, synthetic construct
  REGION 1..356: note = Amino acid sequence of tNlsiaT delta N23AA
MFDRVNQGERNAVSLLKDKLFNEEGEPVNLIFCYTILQMKVAERIMAQHPGERFYVVLMSENRNEKYDYYFNQIKDKAERAYFFYLPYGLNKSFNFIPTMAELKVKSMLLPKVKRIYLASLEKVSIAAFLSTYPDAEIKTFDDGTNNLIQESSYLGDEFSVNGTIKRNFARMMIGDWSIAKTRNASDEHYTIFKGLKNIMDDGRRKMTYLPLFDASELKAGDETGGTVRILLGSPDKEMKEISEKAAKNFKIQYVAPHPRQTYGLSGVTTLNSPYVIEDYILREIKKNPHTRYEIYTFFSGAALTMKDFPNVHVYALKPASLPEDYWLKPVYALFTQSGIPILTFDDKNQSYGKSK

SEQ ID NO: 7 - DNA, 1059 bp, synthetic construct
  misc_feature 1..1059: note = Base sequence of tNlsiaT delta N27AA
  source 1..1059: mol_type = other DNA
atgaaccagggtgaacgcaatgctgttagcctgctgaaagacaaactgtttaacgaagaaggcgaaccggtgaatctgatcttctgttataccattctgcagatgaaagttgcagaacgtattatggctcaacatccgggtgaacgcttttacgtggttctgatgtctgaaaaccgtaacgaaaaatacgattactacttcaaccaaatcaaagacaaagcagaacgcgcttatttcttttatctgccgtacggtctgaacaaaagcttcaacttcatcccgaccatggcagaactgaaagtcaaatctatgctgctgccgaaagtgaaacgtatctacctggcgtcactggaaaaagtgtcgattgcggcctttctgtcaacctatccggatgccgaaatcaaaaccttcgatgacggcacgaacaatctgattcaggaaagctcttatctgggcgatgaattttcggttaacggtacgatcaaacgtaatttcgcccgcatgatgatcggtgattggagtattgcgaaaacccgcaacgcctccgacgaacattacacgatcttcaaaggcctgaaaaacatcatggatgacggtcgtcgcaaaatgacctatctgccgctgttcgatgcaagcgaactgaaagctggcgacgaaaccggcggtacggtccgtattctgctgggttcaccggataaagaaatgaaagaaatctcggaaaaagcagctaaaaacttcaaaatccagtacgttgcgccgcacccgcgccaaacctatggtctgagcggtgttaccacgctgaactctccgtacgtcattgaagattacatcctgcgtgaaattaagaaaaacccgcatacccgctacgaaatctatacgtttttcagcggcgcggccctgacgatgaaagattttccgaacgtccacgtgtatgcgctgaaaccggccagtctgccggaagactactggctgaaaccggtgtatgccctgtttacccagtccggcattccgatcctgacgttcgatgacaaaaaccaaagttacggtaaatccaaataa

SEQ ID NO: 8 - protein, 352 aa, synthetic construct
  REGION 1..352: note = Amino acid sequence of tNlsiaT delta N27AA
MNQGERNAVSLLKDKLFNEEGEPVNLIFCYTILQMKVAERIMAQHPGERFYVVLMSENRNEKYDYYFNQIKDKAERAYFFYLPYGLNKSFNFIPTMAELKVKSMLLPKVKRIYLASLEKVSIAAFLSTYPDAEIKTFDDGTNNLIQESSYLGDEFSVNGTIKRNFARMMIGDWSIAKTRNASDEHYTIFKGLKNIMDDGRRKMTYLPLFDASELKAGDETGGTVRILLGSPDKEMKEISEKAAKNFKIQYVAPHPRQTYGLSGVTTLNSPYVIEDYILREIKKNPHTRYEIYTFFSGAALTMKDFPNVHVYALKPASLPEDYWLKPVYALFTQSGIPILTFDDKNQSYGKSK

SEQ ID NO: 9 - DNA, 1029 bp, synthetic construct
  misc_feature 1..1029: note = Base sequence of tNlsiaT delta N37AA
  source 1..1029: mol_type = other DNA
atgctgaaagacaaactgtttaacgaagaaggcgaaccggtgaatctgatcttctgttataccattctgcagatgaaagttgcagaacgtattatggctcaacatccgggtgaacgcttttacgtggttctgatgtctgaaaaccgtaacgaaaaatacgattactacttcaaccaaatcaaagacaaagcagaacgcgcttatttcttttatctgccgtacggtctgaacaaaagcttcaacttcatcccgaccatggcagaactgaaagtcaaatctatgctgctgccgaaagtgaaacgtatctacctggcgtcactggaaaaagtgtcgattgcggcctttctgtcaacctatccggatgccgaaatcaaaaccttcgatgacggcacgaacaatctgattcaggaaagctcttatctgggcgatgaattttcggttaacggtacgatcaaacgtaatttcgcccgcatgatgatcggtgattggagtattgcgaaaacccgcaacgcctccgacgaacattacacgatcttcaaaggcctgaaaaacatcatggatgacggtcgtcgcaaaatgacctatctgccgctgttcgatgcaagcgaactgaaagctggcgacgaaaccggcggtacggtccgtattctgctgggttcaccggataaagaaatgaaagaaatctcggaaaaagcagctaaaaacttcaaaatccagtacgttgcgccgcacccgcgccaaacctatggtctgagcggtgttaccacgctgaactctccgtacgtcattgaagattacatcctgcgtgaaattaagaaaaacccgcatacccgctacgaaatctatacgtttttcagcggcgcggccctgacgatgaaagattttccgaacgtccacgtgtatgcgctgaaaccggccagtctgccggaagactactggctgaaaccggtgtatgccctgtttacccagtccggcattccgatcctgacgttcgatgacaaaaaccaaagttacggtaaatccaaataa

SEQ ID NO: 10 - protein, 342 aa, synthetic construct
  REGION 1..342: note = Amino acid sequence of tNlsiaT delta N37AA
MLKDKLFNEEGEPVNLIFCYTILQMKVAERIMAQHPGERFYVVLMSENRNEKYDYYFNQIKDKAERAYFFYLPYGLNKSFNFIPTMAELKVKSMLLPKVKRIYLASLEKVSIAAFLSTYPDAEIKTFDDGTNNLIQESSYLGDEFSVNGTIKRNFARMMIGDWSIAKTRNASDEHYTIFKGLKNIMDDGRRKMTYLPLFDASELKAGDETGGTVRILLGSPDKEMKEISEKAAKNFKIQYVAPHPRQTYGLSGVTTLNSPYVIEDYILREIKKNPHTRYEIYTFFSGAALTMKDFPNVHVYALKPASLPEDYWLKPVYALFTQSGIPILTFDDKNQSYGKSK

SEQ ID NO: 11 - DNA, 855 bp, Escherichia coli
  source 1..855: mol_type = genomic DNA; strain = BW25113
atggtactgatgatcgtcagcggacgttcaggttcaggtaaatctgtcgccctgcgtgcgctggaagatatgggtttttactgcgtggataaccttcccgtagtgttgttacccgatctggctcgaactctggccgatcgcgagatttctgccgccgtcagcattgatgttcgtaatatgccggagtcaccagaaatattcgaacaggcgatgagtaacctgcctgacgctttctcaccgcaactcctgttcctggatgccgaccgtaataccttaattcgtcgttacagtgacacgcgccgactgcatccgctttccagcaaaaacctgtcgctggaaagtgctatcgacaaagaaagcgatttgctggaacctctgcgttcgcgagcggatctgattgtcgatacctcagaaatgtccgttcacgagctggctgaaatgctgcgtacccgtctgctgggtaaacgtgaacgcgaactgacaatggtctttgagtctttcggcttcaaacacggtatccctatcgatgcagattacgtctttgacgtgcgcttcttgccgaacccgcactgggatccgaaactgcgtccaatgacaggtcttgataagcccgtcgccgcgttcctcgaccgccacacagaagtacacaattttatctaccagacgcgaagctatcttgagctatggttacctatgctggaaaccaacaaccgtagctacctgacggtcgccattggttgtaccggcgggaagcaccgttcggtgtatattgcagagcaactggcagactacttccgctcgcgcggtaaaaacgtccagtcacgccatcgtacgctggaaaaacgtaaaccatga

SEQ ID NO: 12 - DNA, 3075 bp, Escherichia coli
  source 1..3075: mol_type = genomic DNA; strain = BW25113
atgaccatgattacggattcactggccgtcgttttacaacgtcgtgactgggaaaaccctggcgttacccaacttaatcgccttgcagcacatccccctttcgccagctggcgtaatagcgaagaggcccgcaccgatcgcccttcccaacagttgcgcagcctgaatggcgaatggcgctttgcctggtttccggcaccagaagcggtgccggaaagctggctggagtgcgatcttcctgaggccgatactgtcgtcgtcccctcaaactggcagatgcacggttacgatgcgcccatctacaccaacgtgacctatcccattacggtcaatccgccgtttgttcccacggagaatccgacgggttgttactcgctcacatttaatgttgatgaaagctggctacaggaaggccagacgcgaattatttttgatggcgttaactcggcgtttcatctgtggtgcaacgggcgctgggtcggttacggccaggacagtcgtttgccgtctgaatttgacctgagcgcatttttacgcgccggagaaaaccgcctcgcggtgatggtgctgcgctggagtgacggcagttatctggaagatcaggatatgtggcggatgagcggcattttccgtgacgtctcgttgctgcataaaccgactacacaaatcagcgatttccatgttgccactcgctttaatgatgatttcagccgcgctgtactggaggctgaagttcagatgtgcggcgagttgcgtgactacctacgggtaacagtttctttatggcagggtgaaacgcaggtcgccagcggcaccgcgcctttcggcggtgaaattatcgatgagcgtggtggttatgccgatcgcgtcacactacgtctgaacgtcgaaaacccgaaactgtggagcgccgaaatcccgaatctctatcgtgcggtggttgaactgcacaccgccgacggcacgctgattgaagcagaagcctgcgatgtcggtttccgcgaggtgcggattgaaaatggtctgctgctgctgaacggcaagccgttgctgattcgaggcgttaaccgtcacgagcatcatcctctgcatggtcaggtcatggatgagcagacgatggtgcaggatatcctgctgatgaagcagaacaactttaacgccgtgcgctgttcgcattatccgaaccatccgctgtggtacacgctgtgcgaccgctacggcctgtatgtggtggatgaagccaatattgaaacccacggcatggtgccaatgaatcgtctgaccgatgatccgcgctggctaccggcgatgagcgaacgcgtaacgcgaatggtgcagcgcgatcgtaatcacccgagtgtgatcatctggtcgctggggaatgaatcaggccacggcgctaatcacgacgcgctgtatcgctggatcaaatctgtcgatccttcccgcccggtgcagtatgaaggcggcggagccgacaccacggccaccgatattatttgcccgatgtacgcgcgcgtggatgaagaccagcccttcccggctgtgccgaaatggtccatcaaaaaatggctttcgctacctggagagacgcgcccgctgatcctttgcgaatacgcccacgcgatgggtaacagtcttggcggtttcgctaaatactggcaggcgtttcgtcagtatccccgtttacagggcggcttcgtctgggactgggtggatcagtcgctgattaaatatgatgaaaacggcaacccgtggtcggcttacggcggtgattttggcgatacgccgaacgatcgccagttctgtatgaacggtctggtctttgccgaccgcacgccgcatccagcgctgacggaagcaaaacaccagcagcagtttttccagttccgtttatccgggcaaaccatcgaagtgaccagcgaatacctgttccgtcatagcgataacgagctcctgcactggatggtggcgctggatggtaagccgctggcaagcggtgaagtgcctctggatgtcgctccacaaggtaaacagttgattgaactgcctgaactaccgcagccggagagcgccgggcaactctggctcacagtacgcgtagtgcaaccgaacgcgaccgcatggtcagaagccgggcacatcagcgcctggcagcagtggcgtctggcggaaaacctcagtgtgacgctccccgccgcgtcccacgccatcccgcatctgaccaccagcgaaatggatttttgcatcgagctgggtaataagcgttggcaatttaaccgccagtcaggctttctttcacagatgtggattggcgataaaaaacaactgctgacgccgctgcgcgatcagttcacccgtgcaccgctggataacgacattggcgtaagtgaagcgacccgcattgaccctaacgcctgggtcgaacgctggaaggcggcgggccattaccaggccgaagcagcgttgttgcagtgcacggcagatacacttgctgatgcggtgctgattacgaccgctcacgcgtggcagcatcaggggaaaaccttatttatcagccggaaaacctaccggattgatggtagtggtcaaatggcgattaccgttgatgttgaagtggcgagcgatacaccgcatccggcgcggattggcctgaactgccagctggcgcaggtagcagagcgggtaaactggctcggattagggccgcaagaaaactatcccgaccgccttactgccgcctgttttgaccgctgggatctgccattgtcagacatgtataccccgtacgtcttcccgagcgaaaacggtctgcgctgcgggacgcgcgaattgaattatggcccacaccagtggcgcggcgacttccagttcaacatcagccgctacagtcaacagcaactgatggaaaccagccatcgccatctgctgcacgcggaagaaggcacatggctgaatatcgacggtttccatatggggattggtggcgacgactcctggagcccgtcagtatcggcggaattccagctgagcgccggtcgctaccattaccagttggtctggtgtcaaaaataa

SEQ ID NO: 13 - DNA, 792 bp, Escherichia coli
  source 1..792: mol_type = genomic DNA; strain = BW25113
atgggccttatgaacgcatttgattcgcaaaccgaagattcttcacctgcaattggtcgcaacttgcgtagccgcccgctggcgcgtaaaaaactctccgaaatggtggaagaagagctggaacagatgatccgccgtcgtgaatttggcgaaggtgaacaattaccgtctgaacgcgaactgatggcgttctttaacgtcgggcgtccttctgtgcgcgaagcgctggcagcgttaaaacgcaaaggtctggtgcaaataaacaacggcgaacgcgctcgcgtctcgcgtccttctgcggacactatcatcggtgagctttccggcatggcgaaagatttcctttctcatcctggtgggattgcccatttcgaacaattacgtctgttctttgaatccagcctggtgcgctatgcggctgaacacgccaccgatgagcaaatcgatttgctggcaaaagcactggaaatcaacagtcagtcgctggataacaacgcggcattcattcgttcagacgttgatttccaccgcgtgctggcggagatcccaggtaacccaatcttcatggcgatccacgttgccctgctcgactggctaatcgccgcacgtccaaccgtggctgatcaggctctgcacgagcataacaacgttagctatcaacagcatattgcgatcgttgacgcgatccgccgccacgatcctgacgaagccgatcgtgcgttgcaatcgcatctcaacagcgtctctgctacctggcacgccttcggtcagaccaccaacaaaaagaaataa

SEQ ID NO: 14 - DNA, 894 bp, Escherichia coli
  source 1..894: mol_type = genomic DNA; strain = BW25113
atggcaacgaatttacgtggcgtaatggctgcactcctgactccttttgaccaacaacaagcactggataaagcgagtctgcgtcgcctggttcagttcaatattcagcagggcatcgacggtttatacgtgggtggttcgaccggcgaggcctttgtacaaagcctttccgagcgtgaacaggtactggaaatcgtcgccgaagaggcgaaaggtcagattaaactcatcgcccacgtcggttgcgtcagcaccgccgaaagccaacaacttgcggcatcggctaaacgttatggcttcgatgccgtctccgccgtcacgccgttctactatcctttcagctttgaagagcactgcgatcactatcgggcaattattgattcggcggatggtttgccgatggtggtgtacaacattccagccctgagtggggtaaaactgaccctggatcagatcaacacacttgttacgttgcctggcgtaggtgcgctgaaacagacctctggcgatctctatcagatggagcagatccgtcgtgaacatcctgatctggtgctctataacggttacgacgaaatcttcgcctctggtcttctggcgggcgctgatggtggtatcggtagtacctacaacatcatgggctggcgttatcaggggattgtgaaggcgctgaaagaaggcgatatccagaccgcgcagaagctgcaaaccgaatgtaataaagtcattgatttactgatcaaaacgggcgtattccgcggcctgaaaactgtcctgcattatatggatgtcgtttctgtgccgctgtgccgcaaaccgtttggtccggtagatgaaaaatatctgccagaactgaaggcgctggcccagcagttgatgcaagagcgcgggtga

SEQ ID NO: 15 - DNA, 1491 bp, Escherichia coli
  source 1..1491: mol_type = genomic DNA; strain = BW25113
atgagtactacaacccagaatatcccgtggtatcgccatctcaatcgtgcacaatggcgggcattttccgctgcctggttgggatatctgcttgacggttttgatttcgttttaatcgccctggtactcaccgaagtacagggtgaattcgggctgacgacggtgcaggcggcaagtctgatctccgcagcctttatctctcgctggttcggcggcctgatgctcggcgctatgggtgaccgctacgggcgtcgtctggcaatggtcaccagcatcgttctcttctcggccgggacgctggcctgcggctttgcgccaggctacatcaccatgtttatcgctcgtctggtcatcggcatggggatggcgggtgaatacggttccagcgccacctatgtcattgaaagctggccaaaacatctgcgtaacaaagccagtggttttttgatttcaggcttctctgtgggggccgtcgttgccgctcaggtctatagcctggtggttccggtctggggttggcgtgcgctgttctttatcggcattttgccaatcatctttgctctctggctgcgtaaaaacatcccggaagcggaagactggaaagagaaacacgcaggtaaagcaccagtacgcacaatggtggatattctctaccgtggtgaacatcgcattgccaatatcgtaatgacactggcggcggctactgcgctgtggttctgcttcgccggtaacctgcaaaatgctgcaatcgtcgctgttctcgggctgttatgcgccgcaatctttatcagctttatggtgcaaagtacgggtaaacgctggccaacgggcgtaatgctgatggtggtcgtgttgtttgctttcctctactcatggccgattcaggcgctgctgccaacgtatctgaaaaccgatctggcttataacccgcatactgtcgccaatgtgctgttctttagtggctttggcgcggccgtgggatgctgcgtaggtggcttcctcggtgactggctgggaacccgcaaagcgtacgtttgtagcctgctggcctcgcagctgctgattattccggtatttgcgattggcggcgcaaacgtctgggtgctcggtctgttactgttcttccagcaaatgcttggacaagggatcgccgggatcttaccgaaactgattggcggttatttcgataccgaccagcgtgcagcgggcctgggctttacctacaacgttggcgcattgggcggcgcactggccccaatcatcggcgcgttgatcgctcaacgtctggatctgggtactgcgctggcatcgctctcgttcagtctgacgttcgtggtgatcctgctgattggtctggatatgccttcccgcgttcagcgttggctgcgcccggaagcattgcgtactcatgacgctatcgacggcaaaccatttagcggtgccgtgccatttggcagcgccaaaaacgatttagtcaaaaccaaaagttaa

SEQ ID NO: 16 - DNA, 690 bp, Escherichia coli
  source 1..690: mol_type = genomic DNA; strain = BW25113
atgtcgttacttgcacaactggatcaaaaaatcgctgctaacggtggcctgattgtctcctgccagccggttccggacagtccgctcgataaacccgaaatcgtcgccgccatggcattagcggcagagcaggcgggcgcggttgccattcgcattgaaggtgtggcaaatctgcaagccacgcgtgcggtggtgagcgtgccaattatcgggattgtgaaacgcgatctggaggattctccggtacgcatcacggcctatattgaagatgtcgatgcgctggcgcaggcgggcgcggacattatcgccattgacggcaccgaccgcccgcgtccggtgcctgttgaaacgctgctggcacgtattcaccatcacggtttactggcgatgaccgactgctcaacgccggaagacggcctggcatgccaaaagctgggagccgaaattattggcactacgctttctggctataccacgcctgaaacgccagaagagccggatctggcgctggtgaaaacgttgagcgacgccggatgtcgggtgattgccgaagggcgttacaacacgcctgctcaggcggcagacgcaatgcgccacggcgcgtgggcggtgacggtcggttctgccattacgcgtcttgaacacatttgtcagtggtacaacacagcgatgaaaaaggcggtgctatga

SEQ ID NO: 17 - DNA, 876 bp, Escherichia coli
  source 1..876: mol_type = genomic DNA; strain = BW25113
atgaccacactggcgattgatatcggcggtactaaacttgccgccgcgctgattggcgctgacgggcagatccgcgatcgtcgtgaacttcctacgccagccagccagacaccagaagccttgcgtgatgccttatccgcattagtctctccgttgcaagctcatgcgcagcgggttgccatcgcttcaaccggaattattcgcgacggcagtttgctagcgctgaatccgcataatctcggtggattgctacactttccgttagtcaaaacgctggaacaacttaccaatttgccgaccattgccattaacgacgcgcaggccgcagcatgggcagagtatcaggcgctggaaggcgatataaccgatatggtctttatcaccgtttccactggcgtcggcggcggtgtagtgagcggcggcaaactgcttaccggccctggcggtctggcggggcacatcgggcatacgcttgccgatccacacggcccagtctgcggctgtggacgcacaggttgcgtggaagcaattgcttctggtcgcggcattgcggcggcagcgcagggcgagctggctggcgcggatgctagaactattttcacacgcgccgggcagggcgatgagcaggcgcagcaactgattcatctctccgcacgtacgcttgcaaggctgatcgctgatattaaagccacaactgattgccagtgcgtggtggttggtggcagcgttggtctggcagaagggtatctggcgttggtggaaatgtatctggcgcaggagccagcggcatttcatgttgatttactggcggcgcactaccgccacgatgcaggtttacttggggctgcgctgttggcccagggagaaaaattatga

SEQ ID NO: 18 - DNA, 1041 bp, Campylobacter jejuni
  source 1..1041: mol_type = genomic DNA; strain = ATCC43438
atgaaagaaataaaaatacaaaatataatcataagtgaagaaaaagcacccttagtcgtgcctgaaataggcattaatcataatggcagtttagaactagctaaaattatggtagatgcagcctttagcgcaggtgctaagattataaagcatcaaacccacatcgttgaagatgagatgagtaaggccgctaaaaaagtaattcctggtaatgcaaaaataagcatttatgagattatgcaaaaatgtgctttagattataaagatgagctagcacttaaagaatacacagaaaaattaggtcttgtttatcttagcacacctttttctcgtgcaggtgcaaaccgcttagaagatatgggagttagtgcttttaagattggttcaggtgagtgtaataattatccgcttattaaacacatagcagcctttaaaaagcctatgatagttagcacaggaatgaatagtattgaaagtataaaaccaactgtaaaaatcttattagacaatgaaattccctttgttttaatgcacacgaccaatctttacccaaccccacataatcttgtaagattaaacgctatgcttgaattaaaaaaagaattttcttgcatggtaggcttaagcgaccacacaacagataatcttgcgtgtttaggtgcggttgcacttggtgcttgtgtgcttgaaagacattttactgatagtatggatagaagtggccctgatatagtttgttctatggatacaaaggctttaaaagagctaattatgcaaagtgagcaaatggctataatgagaggaaataatgaaagcaaaaaagcagctaagcaagaacaagttacaattgattttgcctttgcaagcgtagttagtattaaagatattaaaaaaggcgaagttttatctatggacaatatctgggttaaaagacctggacttggtggaattagtgcggttgaatttgaaaatattttaggcaaaaaagcattaagagatatagaaaatgatactcagttaagctatgaggattttgcgtga

SEQ ID NO: 19 - DNA, 1125 bp, Flavobacterium psychrophilum
  source 1..1125: mol_type = genomic DNA; strain = NBRC100250
atgaacaaaaaaattctatttctaacaggaactcgtgccgattttggtaaaataaaatccttaattcaaatcttagaagcccatcccaacttcgaaccctatatttttgtaacagggatgcaccttcaagaagaatatggctatacttttttagaagtacaacgttgcggttttcgcaacattcatacttttcaaaaccatacccacgaaaccacgatggatttaactttggccaaaaccatcacaggattatccgcctatgtaaaagattgccaaccagacatgattgtcatacatggcgatagagtagaagcattagcgggggcaattgtaggttccttaaacaatattttagtgtcccacatagaaggaggcgaagtttcaggaacaatcgatgaattaatacgtcatgctaccagcaaaatgagtcacatacatttcgtatctaatgaccaagccaaaaaaagattacttcaaatgggagaactacacgaatctatctttatcattggttcgcccgatgtagatatcatgttttcaaaaagtttgcccgatttacaaaccgccaaaaaatattacgaaattaccttcaatgattatgccgtggtcatgtttcatcccgtaacaacagaagccaaatatatagcacaatatgccaacgattttgttcatgttttgctagcagatacccacaattacgtagtagtttttcccaacaacgatctaggaagtcatgccattatacaagcctacgaaaaactaaaaaacaacaagcgttttagagtattcccttccttgcgtttcgaatattttttaaccctactaaaaaacgctcaatttattataggaaacagtagtgccggaattcgagaagcaccttattacggattacctattattaatataggaacccgccaacaaaacagagcagcccatactcatattatcaatgtagattacaacaagttgcatatccaagaagcattgtctagcatcgattctcacaaggtacagccttctaaaaatgatttcggacaaggaaatagcgcaaaattattcttagcatctctagaaaaaaatgacatttggcaaataaattaccaaaaacaatttaacgatatataa

SEQ ID NO: 20 - DNA, 672 bp, Pasteurella multocida
  source 1..672: mol_type = genomic DNA; strain = Pm70 ATCC BAA-1909; sub_species = multocida
atgacaaatattgcgatcattcctgcacgagccggctcaaaagggattccagataaaaacctgcagcccgtgggtgggcattctctgattggacgtgctattttagcggcaaaaaatgctgacgttttcgatatgattgtcgtaacctctgatggtgataatatcttacgtgaagcagaaaaatatggggcattagcgctgaaaagacccgctgagttggcccaagacaattcaagaaccattgatgccattttacatgcactagagagcttaaatattcgcgaaggcacttgtaccctattacaaccgactagcccattacgtgatcatttagatatcaaaaatgcgatggatatgtatgtcaatggcggagtacattctgtggtgtcggcgtgcgagtgtgaacatcatccctataaagcttttgcattaagcaaagatcatgaagttttgcctgtacgtgaaattgctgattttgaagccgcacgccaaactttaccgaaaatgtatcgtgcaaatggtgccatttatattaatgacattgcacaattgctaaaagaaaaatatttcttcattccgcctctcaaattctacttaatgccaacttatcgttctgtggatattgatgtgaagcaggatttagaactcgcggaaattttatccaataaatga

SEQ ID NO: 21 - DNA, 20 bp, synthetic construct
  misc_feature 1..20: note = Base sequence of primer Fw for amplification of cat fragment
  source 1..20: mol_type = other DNA
accaggcgtttaagggcacc

SEQ ID NO: 22 - DNA, 45 bp, synthetic construct
  misc_feature 1..45: note = Base sequence of primer Rv for amplification of cat fragment
  source 1..45: mol_type = other DNA
gactacgggcctaaagtcgacagaataaataaatcctggtgtccc

SEQ ID NO: 23 - DNA, 28 bp, synthetic construct
  misc_feature 1..28: note = Base sequence of primer Fw for amplification of sacB fragment
  source 1..28: mol_type = other DNA
gtcgactttaggcccgtagtctgcaaat

SEQ ID NO: 24 - DNA, 21 bp, synthetic construct
  misc_feature 1..21: note = Base sequence of primer Rv for amplification of sacB fragment
  source 1..21: mol_type = other DNA
tacggttagccatttgcctgc

SEQ ID NO: 25 - DNA, 20 bp, synthetic construct
  misc_feature 1..20: note = Base sequence of Primer Fw for amplification of lacZ upstream 1 fragment
  source 1..20: mol_type = other DNA
tctcccatgaagacggtacg

SEQ ID NO: 26 - DNA, 37 bp, synthetic construct
  misc_feature 1..37: note = Base sequence of Primer Rv for amplification of lacZ upstream 1 fragment
  source 1..37: mol_type = other DNA
aataagtgcggccgcagctgtttcctgtgtgaaattg

SEQ ID NO: 27 - DNA, 33 bp, synthetic construct
  misc_feature 1..33: note = Base sequence of Primer Fw for amplification of lacZ downstream 1 fragment
  source 1..33: mol_type = other DNA
ccgatatgcggccgctaataaccgggcaggcca

SEQ ID NO: 28 - DNA, 20 bp, synthetic construct
  misc_feature 1..20: note = Base sequence of Primer Rv for amplification of lacZ downstream 1 fragment
  source 1..20: mol_type = other DNA
ttcaccggtagcaaagaacg

SEQ ID NO: 29 - DNA, 20 bp, synthetic construct
  misc_feature 1..20: note = Base sequence of Primer Fw for amplification of lacZ upstream 2 fragment
  source 1..20: mol_type = other DNA
tctcccatgaagacggtacg

SEQ ID NO: 30 - DNA, 37 bp, synthetic construct
  misc_feature 1..37: note = Base sequence of Primer Rv for amplification of lacZ upstream 2 fragment
  source 1..37: mol_type = other DNA
cctgcccggttattaagctgtttcctgtgtgaaattg

SEQ ID NO: 31 - DNA, 33 bp, synthetic construct
  misc_feature 1..33: note = Base sequence of Primer Fw for amplification of lacZ downstream 2 fragment
  source 1..33: mol_type = other DNA
acacaggaaacagcttaataaccgggcaggcca

SEQ ID NO: 32 - DNA, 20 bp, synthetic construct
  misc_feature 1..20: note = Base sequence of Primer Rv for amplification of lacZ downstream 2 fragment
  source 1..20: mol_type = other DNA
ttcaccggtagcaaagaacg

SEQ ID NO: 33 - DNA, 20 bp, synthetic construct
  misc_feature 1..20: note = Primer Fw for making fragments for disrupting lacZ
  source 1..20: mol_type = other DNA
ctcgcaatcaaattcagccg

SEQ ID NO: 34 - DNA, 19 bp, synthetic construct
  misc_feature 1..19: note = Primer Rv for making fragments for disrupting lacZ
  source 1..19: mol_type = other DNA
gctgtctgaacagttccag

SEQ ID NO: 35 - DNA, 21 bp, synthetic construct
  misc_feature 1..21: note = Base sequence of Primer Fw for amplification of nanR upstream 1 fragment
  source 1..21: mol_type = other DNA
ggaaataaggtgaccatcagc

SEQ ID NO: 36 - DNA, 35 bp, synthetic construct
  misc_feature 1..35: note = Base sequence of Primer Rv for amplification of nanR upstream 1 fragment
  source 1..35: mol_type = other DNA
aataagtgcggccgctctgtaaggtcagtgtgatt

SEQ ID NO: 37 - DNA, 34 bp, synthetic construct
  misc_feature 1..34: note = Base sequence of Primer Fw for amplification of nanK downstream 1 fragment
  source 1..34: mol_type = other DNA
ccgatatgcggccgctgatgggtgaagtacagtc

SEQ ID NO: 38 - DNA, 20 bp, synthetic construct
  misc_feature 1..20: note = Base sequence of Primer Rv for amplification of nanK downstream 1 fragment
  source 1..20: mol_type = other DNA
tcgacctgctgtttttccac

SEQ ID NO: 39 - DNA, 21 bp, synthetic construct
  misc_feature 1..21: note = Base sequence of Primer Fw for amplification of nanR upstream 2 fragment
  source 1..21: mol_type = other DNA
ggaaataaggtgaccatcagc

SEQ ID NO: 40 - DNA, 35 bp, synthetic construct
  misc_feature 1..35: note = Base sequence of Primer Rv for amplification of nanR upstream 2 fragment
  source 1..35: mol_type = other DNA
gtacttcacccatcatctgtaaggtcagtgtgatt

SEQ ID NO: 41 - DNA, 34 bp, synthetic construct
  misc_feature 1..34: note = Base sequence of Primer Fw for amplification of nanK downstream 2 fragment
  source 1..34: mol_type = other DNA
cactgaccttacagatgatgggtgaagtacagtc

SEQ ID NO: 42 - DNA, 20 bp, synthetic construct
  misc_feature 1..20: note = Base sequence of Primer Rv for amplification of nanK downstream 2 fragment
  source 1..20: mol_type = other DNA
tcgacctgctgtttttccac

SEQ ID NO: 43 - DNA, 20 bp, synthetic construct
  misc_feature 1..20: note = Primer Fw for making fragments for disrupting nanRATEK
  source 1..20: mol_type = other DNA
gagcgaatgagttttaacgg

SEQ ID NO: 44 - DNA, 20 bp, synthetic construct
  misc_feature 1..20: note = Primer Rv for making fragments for disrupting nanRATEK
  source 1..20: mol_type = other DNA
caaagagcactggacgctac

SEQ ID NO: 45 - DNA, 34 bp, synthetic construct
  misc_feature 1..34: note = Base sequence of Primer Fw for amplification of CjneuB fragment
  source 1..34: mol_type = other DNA
cacaggaaacagaccatgaaagaaataaaaatac

SEQ ID NO: 46 - DNA, 35 bp, synthetic construct
  misc_feature 1..35: note = Base sequence of Primer Rv for amplification of CjneuB fragment
  source 1..35: mol_type = other DNA
aatttttttgttcatggtctgtttcctgtcacgca

SEQ ID NO: 47 - DNA, 29 bp, synthetic construct
  misc_feature 1..29: note = Base sequence of Primer Fw for amplification of FpneuC fragment
  source 1..29: mol_type = other DNA
atgaacaaaaaaattctatttctaacagg

SEQ ID NO: 48 - DNA, 40 bp, synthetic construct
  misc_feature 1..40: note = Base sequence of Primer Rv for amplification of FpneuC fragment
  source 1..40: mol_type = other DNA
ggatccccgggtaccttatatatcgttaaattgtttttgg

SEQ ID NO: 49 - DNA, 28 bp, synthetic construct
  misc_feature 1..28: note = Base sequence of Primer Fw for amplification of NlsiaT
  source 1..28: mol_type = other DNA
ccatgattacatgggcctgaagaaagcg

SEQ ID NO: 50 - DNA, 35 bp, synthetic construct
  misc_feature 1..35: note = Base sequence of Primer Rv for amplification of NlsiaT
  source 1..35: mol_type = other DNA
tcataataagctcctttatttggatttaccgtaac

SEQ ID NO: 51 - DNA, 34 bp, synthetic construct
  misc_feature 1..34: note = Base sequence of Primer Fw for amplification of tNlsiaT delta N20AA
  source 1..34: mol_type = other DNA
ccatgattacatgttttatacgttcgatcgtgtg

SEQ ID NO: 52 - DNA, 34 bp, synthetic construct
  misc_feature 1..34: note = Base sequence of Primer Fw for amplification of tNlsiaT delta N23AA
  source 1..34: mol_type = other DNA
tatgaccatgattacatgttcgatcgtgtgaacc

SEQ ID NO: 53 - DNA, 32 bp, synthetic construct
  misc_feature 1..32: note = Base sequence of Primer Fw for amplification of tNlsiaT delta N27AA
  source 1..32: mol_type = other DNA
ccatgattacatgaaccagggtgaacgcaatg

SEQ ID NO: 54 - DNA, 34 bp, synthetic construct
  misc_feature 1..34: note = Base sequence of Primer Fw for amplification of tNlsiaT delta N37AA
  source 1..34: mol_type = other DNA
ccatgattacatgctgaaagacaaactgtttaac

SEQ ID NO: 55 - DNA, 34 bp, synthetic construct
  misc_feature 1..34: note = Base sequence of Primer Fw for amplification of PmneuA
  source 1..34: mol_type = other DNA
aggagcttattatgacaaatattgcgatcattcc

SEQ ID NO: 56 - DNA, 38 bp, synthetic construct
  misc_feature 1..38: note = Base sequence of Primer Rv for amplification of PmneuA
  source 1..38: mol_type = other DNA
aaaacgacggccagttcatttattggataaaatttccg